European Patent Application EP 4 279 511 A2, published November 22, 2023. Title: Cytotoxicity-inducing therapeutic agent. Applicant: CHUGAI SEIYAKU KABUSHIKI KAISHA. Application EP. The sequence listing filed with the application follows.

SEQUENCE LISTING (92 sequences)

SEQ ID NO: 1 - DNA, 1812 bp, Homo sapiens
  source 1..1812: mol_type = unassigned DNA
atggccgggaccgtgcgcaccgcgtgcttggtggtggcgatgctgctcagcttggacttcccgggacaggcgcagcccccgccgccgccgccggacgccacctgtcaccaagtccgctccttcttccagagactgcagcccggactcaagtgggtgccagaaactcccgtgccaggatcagatttgcaagtatgtctccctaagggcccaacatgctgctcaagaaagatggaagaaaaataccaactaacagcacgattgaacatggaacagctgcttcagtctgcaagtatggagctcaagttcttaattattcagaatgctgcggttttccaagaggcctttgaaattgttgttcgccatgccaagaactacaccaatgccatgttcaagaacaactacccaagcctgactccacaagcttttgagtttgtgggtgaatttttcacagatgtgtctctctacatcttgggttctgacatcaatgtagatgacatggtcaatgaattgtttgacagcctgtttccagtcatctatacccagctaatgaacccaggcctgcctgattcagccttggacatcaatgagtgcctccgaggagcaagacgtgacctgaaagtatttgggaatttccccaagcttattatgacccaggtttccaagtcactgcaagtcactaggatcttccttcaggctctgaatcttggaattgaagtgatcaacacaactgatcacctgaagttcagtaaggactgtggccgaatgctcaccagaatgtggtactgctcttactgccagggactgatgatggttaaaccctgtggcggttactgcaatgtggtcatgcaaggctgtatggcaggtgtggtggagattgacaagtactggagagaatacattctgtcccttgaagaacttgtgaatggcatgtacagaatctatgacatggagaacgtactgcttggtctcttttcaacaatccatgattctatccagtatgtccagaagaatgcaggaaagctgaccaccactgaaactgagaagaaaatatggcacttcaaatatcctatcttcttcctgtgtatagggctagacttacagattggcaagttatgtgcccattctcaacaacgccaatatagatctgcttattatcctgaagatctctttattgacaagaaagtattaaaagttgctcatgtagaacatgaagaaaccttatccagccgaagaagggaactaattcagaagttgaagtctttcatcagcttctatagtgctttgcctggctacatctgcagccatagccctgtggcggaaaacgacaccctttgctggaatggacaagaactcgtggagagatacagccaaaaggcagcaaggaatggaatgaaaaaccagttcaatctccatgagctgaaaatgaagggccctgagccagtggtcagtcaaattattgacaaactgaagcacattaaccagctcctgagaaccatgtctatgcccaaaggtagagttctggataaaaacctggatgaggaagggtttgaaagtggagactgcggtgatgatgaagatgagtgcattggaggctctggtgatggaatgataaaagtgaagaatcagctccgcttccttgcagaactggcctatgatctggatgtggatgatgcgcctggaaacagtcagcaggcaactccgaaggacaacgagataagcacctttcacaacctcgggaacgttcattccccgctgaagcttctcaccagcatggccatctcggtggtgtgcttcttcttcctggtgcactga

SEQ ID NO: 2 - protein, 603 aa, Homo sapiens
MAGTVRTACLVVAMLLSLDFPGQAQPPPPPPDATCHQVRSFFQRLQPGLKWVPETPVPGSDLQVCLPKGPTCCSRKMEEKYQLTARLNMEQLLQSASMELKFLIIQNAAVFQEAFEIVVRHAKNYTNAMFKNNYPSLTPQAFEFVGEFFTDVSLYILGSDINVDDMVNELFDSLFPVIYTQLMNPGLPDSALDINECLRGARRDLKVFGNFPKLIMTQVSKSLQVTRIFLQALNLGIEVINTTDHLKFSKDCGRMLTRMWYCSYCQGLMMVKPCGGYCNVVMQGCMAGVVEIDKYWREYILSLEELVNGMYRIYDMENVLLGLFSTIHDSIQYVQKNAGKLTTTETEKKIWHFKYPIFFLCIGLDLQIGKLCAHSQQRQYRSAYYPEDLFIDKKVLKVAHVEHEETLSSRRRELIQKLKSFISFYSALPGYICSHSPVAENDTLCWNGQELVERYSQKAARNGMKNQFNLHELKMKGPEPVVSQIIDKLKHINQLLRTMSMPKGRVLDKNLDEEGFESGDCGDDEDECIGGSGDGMIKVKNQLRFLAELAYDLDVDDAPGNSQQATPKDNEISTFHNLGNVHSPLKLLTSMAISVVCFFFLVH

SEQ ID NO: 3 - DNA, 945 bp, Homo sapiens
  source 1..945: mol_type = unassigned DNA
atggcgcccccgcaggtcctcgcgttcgggcttctgcttgccgcggcgacggcgacttttgccgcagctcaggaagaatgtgtctgtgaaaactacaagctggccgtaaactgctttgtgaataataatcgtcaatgccagtgtacttcagttggtgcacaaaatactgtcatttgctcaaagctggctgccaaatgtttggtgatgaaggcagaaatgaatggctcaaaacttgggagaagagcaaaacctgaaggggccctccagaacaatgatgggctttatgatcctgactgcgatgagagcgggctctttaaggccaagcagtgcaacggcacctccatgtgctggtgtgtgaacactgctggggtcagaagaacagacaaggacactgaaataacctgctctgagcgagtgagaacctactggatcatcattgaactaaaacacaaagcaagagaaaaaccttatgatagtaaaagtttgcggactgcacttcagaaggagatcacaacgcgttatcaactggatccaaaatttatcacgagtattttgtatgagaataatgttatcactattgatctggttcaaaattcttctcaaaaaactcagaatgatgtggacatagctgatgtggcttattattttgaaaaagatgttaaaggtgaatccttgtttcattctaagaaaatggacctgacagtaaatggggaacaactggatctggatcctggtcaaactttaatttattatgttgatgaaaaagcacctgaattctcaatgcagggtctaaaagctggtgttattgctgttattgtggttgtggtgatagcagttgttgctggaattgttgtgctggttatttccagaaagaagagaatggcaaagtatgagaaggctgagataaaggagatgggtgagatgcatagggaactcaatgcataa

SEQ ID NO: 4 - protein, 314 aa, Homo sapiens
MAPPQVLAFGLLLAAATATFAAAQEECVCENYKLAVNCFVNNNRQCQCTSVGAQNTVICSKLAAKCLVMKAEMNGSKLGRRAKPEGALQNNDGLYDPDCDESGLFKAKQCNGTSMCWCVNTAGVRRTDKDTEITCSERVRTYWIIIELKHKAREKPYDSKSLRTALQKEITTRYQLDPKFITSILYENNVITIDLVQNSSQKTQNDVDIADVAYYFEKDVKGESLFHSKKMDLTVNGEQLDLDPGQTLIYYVDEKAPEFSMQGLKAGVIAVIVVVVIAVVAGIVVLVISRKKRMAKYEKAEIKEMGEMHRELNA

SEQ ID NO: 5 - protein, 4 aa, synthetic construct
  REGION 1..4: note = an artificially synthesized sequence
GGGS

SEQ ID NO: 6 - protein, 4 aa, synthetic construct
  REGION 1..4: note = an artificially synthesized sequence
SGGG

SEQ ID NO: 7 - protein, 5 aa, synthetic construct
  REGION 1..5: note = an artificially synthesized sequence
GGGGS

SEQ ID NO: 8 - protein, 5 aa, synthetic construct
  REGION 1..5: note = an artificially synthesized sequence
SGGGG

SEQ ID NO: 9 - protein, 6 aa, synthetic construct
  REGION 1..6: note = an artificially synthesized sequence
GGGGGS

SEQ ID NO: 10 - protein, 6 aa, synthetic construct
  REGION 1..6: note = an artificially synthesized sequence
SGGGGG

SEQ ID NO: 11 - protein, 7 aa, synthetic construct
  REGION 1..7: note = an artificially synthesized sequence
GGGGGGS

SEQ ID NO: 12 - protein, 7 aa, synthetic construct
  REGION 1..7: note = an artificially synthesized sequence
SGGGGGG

SEQ ID NO: 13 - DNA, 1125 bp, Homo sapiens
  source 1..1125: mol_type = unassigned DNA
atgtggttcttgacaactctgctcctttgggttccagttgatgggcaagtggacaccacaaaggcagtgatcactttgcagcctccatgggtcagcgtgttccaagaggaaaccgtaaccttgcactgtgaggtgctccatctgcctgggagcagctctacacagtggtttctcaatggcacagccactcagacctcgacccccagctacagaatcacctctgccagtgtcaatgacagtggtgaatacaggtgccagagaggtctctcagggcgaagtgaccccatacagctggaaatccacagaggctggctactactgcaggtctccagcagagtcttcacggaaggagaacctctggccttgaggtgtcatgcgtggaaggataagctggtgtacaatgtgctttactatcgaaatggcaaagcctttaagtttttccactggaattctaacctcaccattctgaaaaccaacataagtcacaatggcacctaccattgctcaggcatgggaaagcatcgctacacatcagcaggaatatctgtcactgtgaaagagctatttccagctccagtgctgaatgcatctgtgacatccccactcctggaggggaatctggtcaccctgagctgtgaaacaaagttgctcttgcagaggcctggtttgcagctttacttctccttctacatgggcagcaagaccctgcgaggcaggaacacatcctctgaataccaaatactaactgctagaagagaagactctgggttatactggtgcgaggctgccacagaggatggaaatgtccttaagcgcagccctgagttggagcttcaagtgcttggcctccagttaccaactcctgtctggtttcatgtccttttctatctggcagtgggaataatgtttttagtgaacactgttctctgggtgacaatacgtaaagaactgaaaagaaagaaaaagtgggatttagaaatctctttggattctggtcatgagaagaaggtaatttccagccttcaagaagacagacatttagaagaagagctgaaatgtcaggaacaaaaagaagaacagctgcaggaaggggtgcaccggaaggagccccagggggccacgtag

SEQ ID NO: 14 - protein, 374 aa, Homo sapiens
MWFLTTLLLWVPVDGQVDTTKAVITLQPPWVSVFQEETVTLHCEVLHLPGSSSTQWFLNGTATQTSTPSYRITSASVNDSGEYRCQRGLSGRSDPIQLEIHRGWLLLQVSSRVFTEGEPLALRCHAWKDKLVYNVLYYRNGKAFKFFHWNSNLTILKTNISHNGTYHCSGMGKHRYTSAGISVTVKELFPAPVLNASVTSPLLEGNLVTLSCETKLLLQRPGLQLYFSFYMGSKTLRGRNTSSEYQILTARREDSGLYWCEAATEDGNVLKRSPELELQVLGLQLPTPVWFHVLFYLAVGIMFLVNTVLWVTIRKELKRKKKWDLEISLDSGHEKKVISSLQEDRHLEEELKCQEQKEEQLQEGVHRKEPQGAT

SEQ ID NO: 15 - DNA, 951 bp, Homo sapiens
  source 1..951: mol_type = unassigned DNA
atgactatggagacccaaatgtctcagaatgtatgtcccagaaacctgtggctgcttcaaccattgacagttttgctgctgctggcttctgcagacagtcaagctgctcccccaaaggctgtgctgaaacttgagcccccgtggatcaacgtgctccaggaggactctgtgactctgacatgccagggggctcgcagccctgagagcgactccattcagtggttccacaatgggaatctcattcccacccacacgcagcccagctacaggttcaaggccaacaacaatgacagcggggagtacacgtgccagactggccagaccagcctcagcgaccctgtgcatctgactgtgctttccgaatggctggtgctccagacccctcacctggagttccaggagggagaaaccatcatgctgaggtgccacagctggaaggacaagcctctggtcaaggtcacattcttccagaatggaaaatcccagaaattctcccatttggatcccaccttctccatcccacaagcaaaccacagtcacagtggtgattaccactgcacaggaaacataggctacacgctgttctcatccaagcctgtgaccatcactgtccaagtgcccagcatgggcagctcttcaccaatgggggtcattgtggctgtggtcattgcgactgctgtagcagccattgttgctgctgtagtggccttgatctactgcaggaaaaagcggatttcagccaattccactgatcctgtgaaggctgcccaatttgagccacctggacgtcaaatgattgccatcagaaagagacaacttgaagaaaccaacaatgactatgaaacagctgacggcggctacatgactctgaaccccagggcacctactgacgatgataaaaacatctacctgactcttcctcccaacgaccatgtcaacagtaataactaa

SEQ ID NO: 16 - protein, 316 aa, Homo sapiens
MTMETQMSQNVCPRNLWLLQPLTVLLLLASADSQAAPPKAVLKLEPPWINVLQEDSVTLTCQGARSPESDSIQWFHNGNLIPTHTQPSYRFKANNNDSGEYTCQTGQTSLSDPVHLTVLSEWLVLQTPHLEFQEGETIMLRCHSWKDKPLVKVTFFQNGKSQKFSHLDPTFSIPQANHSHSGDYHCTGNIGYTLFSSKPVTITVQVPSMGSSSPMGVIVAVVIATAVAAIVAAVVALIYCRKKRISANSTDPVKAAQFEPPGRQMIAIRKRQLEETNNDYETADGGYMTLNPRAPTDDDKNIYLTLPPNDHVNSNN

SEQ ID NO: 17 - DNA, 876 bp, Homo sapiens
  source 1..876: mol_type = unassigned DNA
atgggaatcctgtcattcttacctgtccttgccactgagagtgactgggctgactgcaagtccccccagccttggggtcatatgcttctgtggacagctgtgctattcctggctcctgttgctgggacacctgcagctcccccaaaggctgtgctgaaactcgagccccagtggatcaacgtgctccaggaggactctgtgactctgacatgccgggggactcacagccctgagagcgactccattcagtggttccacaatgggaatctcattcccacccacacgcagcccagctacaggttcaaggccaacaacaatgacagcggggagtacacgtgccagactggccagaccagcctcagcgaccctgtgcatctgactgtgctttctgagtggctggtgctccagacccctcacctggagttccaggagggagaaaccatcgtgctgaggtgccacagctggaaggacaagcctctggtcaaggtcacattcttccagaatggaaaatccaagaaattttcccgttcggatcccaacttctccatcccacaagcaaaccacagtcacagtggtgattaccactgcacaggaaacataggctacacgctgtactcatccaagcctgtgaccatcactgtccaagctcccagctcttcaccgatggggatcattgtggctgtggtcactgggattgctgtagcggccattgttgctgctgtagtggccttgatctactgcaggaaaaagcggatttcagccaatcccactaatcctgatgaggctgacaaagttggggctgagaacacaatcacctattcacttctcatgcacccggatgctctggaagagcctgatgaccagaaccgtatttag

SEQ ID NO: 18 - protein, 291 aa, Homo sapiens
MGILSFLPVLATESDWADCKSPQPWGHMLLWTAVLFLAPVAGTPAAPPKAVLKLEPQWINVLQEDSVTLTCRGTHSPESDSIQWFHNGNLIPTHTQPSYRFKANNNDSGEYTCQTGQTSLSDPVHLTVLSEWLVLQTPHLEFQEGETIVLRCHSWKDKPLVKVTFFQNGKSKKFSRSDPNFSIPQANHSHSGDYHCTGNIGYTLYSSKPVTITVQAPSSSPMGIIVAVVTGIAVAAIVAAVVALIYCRKKRISANPTNPDEADKVGAENTITYSLLMHPDALEEPDDQNRI

SEQ ID NO: 19 - DNA, 765 bp, Homo sapiens
  source 1..765: mol_type = unassigned DNA
atgtggcagctgctcctcccaactgctctgctacttctagtttcagctggcatgcggactgaagatctcccaaaggctgtggtgttcctggagcctcaatggtacagggtgctcgagaaggacagtgtgactctgaagtgccagggagcctactcccctgaggacaattccacacagtggtttcacaatgagagcctcatctcaagccaggcctcgagctacttcattgacgctgccacagttgacgacagtggagagtacaggtgccagacaaacctctccaccctcagtgacccggtgcagctagaagtccatatcggctggctgttgctccaggcccctcggtgggtgttcaaggaggaagaccctattcacctgaggtgtcacagctggaagaacactgctctgcataaggtcacatatttacagaatggcaaaggcaggaagtattttcatcataattctgacttctacattccaaaagccacactcaaagacagcggctcctacttctgcagggggcttgttgggagtaaaaatgtgtcttcagagactgtgaacatcaccatcactcaaggtttgtcagtgtcaaccatctcatcattctttccacctgggtaccaagtctctttctgcttggtgatggtactcctttttgcagtggacacaggactatatttctctgtgaagacaaacattcgaagctcaacaagagactggaaggaccataaatttaaatggagaaaggaccctcaagacaaatga

SEQ ID NO: 20 - protein, 254 aa, Homo sapiens [sequence omitted]

SEQ ID NO: 21 - DNA, 702 bp, Homo sapiens
  source 1..702: mol_type = unassigned DNA
atgtggcagctgctcctcccaactgctctgctacttctagtttcagctggcatgcggactgaagatctcccaaaggctgtggtgttcctggagcctcaatggtacagcgtgcttgagaaggacagtgtgactctgaagtgccagggagcctactcccctgaggacaattccacacagtggtttcacaatgagagcctcatctcaagccaggcctcgagctacttcattgacgctgccacagtcaacgacagtggagagtacaggtgccagacaaacctctccaccctcagtgacccggtgcagctagaagtccatatcggctggctgttgctccaggcccctcggtgggtgttcaaggaggaagaccctattcacctgaggtgtcacagctggaagaacactgctctgcataaggtcacatatttacagaatggcaaagacaggaagtattttcatcataattctgacttccacattccaaaagccacactcaaagatagcggctcctacttctgcagggggcttgttgggagtaaaaatgtgtcttcagagactgtgaacatcaccatcactcaaggtttggcagtgtcaaccatctcatcattctctccacctgggtaccaagtctctttctgcttggtgatggtactcctttttgcagtggacacaggactatatttctctgtgaagacaaacatttga

SEQ ID NO: 22 - protein, 233 aa, Homo sapiens
MWQLLLPTALLLLVSAGMRTEDLPKAVVFLEPQWYSVLEKDSVTLKCQGAYSPEDNSTQWFHNESLISSQASSYFIDAATVNDSGEYRCQTNLSTLSDPVQLEVHIGWLLLQAPRWVFKEEDPIHLRCHSWKNTALHKVTYLQNGKDRKYFHHNSDFHIPKATLKDSGSYFCRGLVGSKNVSSETVNITITQGLAVSTISSFSPPGYQVSFCLVMVLLFAVDTGLYFSVKTNI

SEQ ID NO: 23 - protein, 330 aa, synthetic construct [sequence omitted]

SEQ ID NO: 24 - protein, 326 aa, synthetic construct
  REGION 1..326: note = an artificially synthesized sequence
ASTKGPSVFPLAPCSRSTSESTAALGCLVKDYFPEPVTVSWNSGALTSGVHTFPAVLQSSGLYSLSSVVTVPSSNFGTQTYTCNVDHKPSNTKVDKTVERKCCVECPPCPAPPVAGPSVFLFPPKPKDTLMISRTPEVTCVVVDVSHEDPEVQFNWYVDGVEVHNAKTKPREEQFNSTFRVVSVLTVVHQDWLNGKEYKCKVSNKGLPAPIEKTISKTKGQPREPQVYTLPPSREEMTKNQVSLTCLVKGFYPSDIAVEWESNGQPENNYKTTPPMLDSDGSFFLYSKLTVDKSRWQQGNVFSCSVMHEALHNHYTQKSLSLSPGK

SEQ ID NO: 25 - protein, 377 aa, synthetic construct
  REGION 1..377: note = an artificially synthesized sequence
ASTKGPSVFPLAPCSRSTSGGTAALGCLVKDYFPEPVTVSWNSGALTSGVHTFPAVLQSSGLYSLSSVVTVPSSSLGTQTYTCNVNHKPSNTKVDKRVELKTPLGDTTHTCPRCPEPKSCDTPPPCPRCPEPKSCDTPPPCPRCPEPKSCDTPPPCPRCPAPELLGGPSVFLFPPKPKDTLMISRTPEVTCVVVDVSHEDPEVQFKWYVDGVEVHNAKTKPREEQYNSTFRVVSVLTVLHQDWLNGKEYKCKVSNKALPAPIEKTISKTKGQPREPQVYTLPPSREEMTKNQVSLTCLVKGFYPSDIAVEWESSGQPENNYNTTPPMLDSDGSFFLYSKLTVDKSRWQQGNIFSCSVMHEALHNRFTQKSLSLSPGK

SEQ ID NO: 26 - protein, 327 aa, synthetic construct
  REGION 1..327: note = an artificially synthesized sequence
ASTKGPSVFPLAPCSRSTSESTAALGCLVKDYFPEPVTVSWNSGALTSGVHTFPAVLQSSGLYSLSSVVTVPSSSLGTKTYTCNVDHKPSNTKVDKRVESKYGPPCPSCPAPEFLGGPSVFLFPPKPKDTLMISRTPEVTCVVVDVSQEDPEVQFNWYVDGVEVHNAKTKPREEQFNSTYRVVSVLTVLHQDWLNGKEYKCKVSNKGLPSSIEKTISKAKGQPREPQVYTLPPSQEEMTKNQVSLTCLVKGFYPSDIAVEWESNGQPENNYKTTPPVLDSDGSFFLYSRLTVDKSRWQEGNVFSCSVMHEALHNHYTQKSLSLSLGK

SEQ ID NO: 27 - DNA, 549 bp, Homo sapiens
  source 1..549: mol_type = unassigned DNA
atggaacaggggaagggcctggctgtcctcatcctggctatcattcttcttcaaggtactttggcccagtcaatcaaaggaaaccacttggttaaggtgtatgactatcaagaagatggttcggtacttctgacttgtgatgcagaagccaaaaatatcacatggtttaaagatgggaagatgatcggcttcctaactgaagataaaaaaaaatggaatctgggaagtaatgccaaggaccctcgagggatgtatcagtgtaaaggatcacagaacaagtcaaaaccactccaagtgtattacagaatgtgtcagaactgcattgaactaaatgcagccaccatatctggctttctctttgctgaaatcgtcagcattttcgtccttgctgttggggtctacttcattgctggacaggatggagttcgccagtcgagagcttcagacaagcagactctgttgcccaatgaccagctctaccagcccctcaaggatcgagaagatgaccagtacagccaccttcaaggaaaccagttgaggaggaattga

SEQ ID NO: 28 - protein, 182 aa, Homo sapiens
MEQGKGLAVLILAIILLQGTLAQSIKGNHLVKVYDYQEDGSVLLTCDAEAKNITWFKDGKMIGFLTEDKKKWNLGSNAKDPRGMYQCKGSQNKSKPLQVYYRMCQNCIELNAATISGFLFAEIVSIFVLAVGVYFIAGQDGVRQSRASDKQTLLPNDQLYQPLKDREDDQYSHLQGNQLRRN

SEQ ID NO: 29 - DNA, 516 bp, Homo sapiens
  source 1..516: mol_type = unassigned DNA
atggaacatagcacgtttctctctggcctggtactggctacccttctctcgcaagtgagccccttcaagatacctatagaggaacttgaggacagagtgtttgtgaattgcaataccagcatcacatgggtagagggaacggtgggaacactgctctcagacattacaagactggacctgggaaaacgcatcctggacccacgaggaatatataggtgtaatgggacagatatatacaaggacaaagaatctaccgtgcaagttcattatcgaatgtgccagagctgtgtggagctggatccagccaccgtggctggcatcattgtcactgatgtcattgccactctgctccttgctttgggagtcttctgctttgctggacatgagactggaaggctgtctggggctgccgacacacaagctctgttgaggaatgaccaggtctatcagcccctccgagatcgagatgatgctcagtacagccaccttggaggaaactgggctcggaacaagtga

SEQ ID NO: 30 - protein, 171 aa, Homo sapiens
MEHSTFLSGLVLATLLSQVSPFKIPIEELEDRVFVNCNTSITWVEGTVGTLLSDITRLDLGKRILDPRGIYRCNGTDIYKDKESTVQVHYRMCQSCVELDPATVAGIIVTDVIATLLLALGVFCFAGHETGRLSGAADTQALLRNDQVYQPLRDRDDAQYSHLGGNWARNK

SEQ ID NO: 31 - DNA, 624 bp, Homo sapiens
  source 1..624: mol_type = unassigned DNA
atgcagtcgggcactcactggagagttctgggcctctgcctcttatcagttggcgtttgggggcaagatggtaatgaagaaatgggtggtattacacagacaccatataaagtctccatctctggaaccacagtaatattgacatgccctcagtatcctggatctgaaatactatggcaacacaatgataaaaacataggcggtgatgaggatgataaaaacataggcagtgatgaggatcacctgtcactgaaggaattttcagaattggagcaaagtggttattatgtctgctaccccagaggaagcaaaccagaagatgcgaacttttatctctacctgagggcaagagtgtgtgagaactgcatggagatggatgtgatgtcggtggccacaattgtcatagtggacatctgcatcactgggggcttgctgctgctggtttactactggagcaagaatagaaaggccaaggccaagcctgtgacacgaggagcgggtgctggcggcaggcaaaggggacaaaacaaggagaggccaccacctgttcccaacccagactatgagcccatccggaaaggccagcgggacctgtattctggcctgaatcagagacgcatctga

SEQ ID NO: 32 - protein, 207 aa, Homo sapiens
MQSGTHWRVLGLCLLSVGVWGQDGNEEMGGITQTPYKVSISGTTVILTCPQYPGSEILWQHNDKNIGGDEDDKNIGSDEDHLSLKEFSELEQSGYYVCYPRGSKPEDANFYLYLRARVCENCMEMDVMSVATIVIVDICITGGLLLLVYYWSKNRKAKAKPVTRGAGAGGRQRGQNKERPPPVPNPDYEPIRKGQRDLYSGLNQRRI

SEQ ID NO: 33 - protein, 523 aa, synthetic construct
  REGION 1..523: note = an artificially synthesized sequence
MGWSCIILFLVATATGVHSQVQLVQSGAEVKKPGASVKVSCKASGYTFTDYEMHWIRQPPGQGLEWIGAIDPKTGDTAYSQKFKGRVTLTADKSTSTAYMELSSLTSEDTAVYYCTRFYSYTYWGQGTLVTVSSGGGGSGGGGSGGGGSDIVMTQSPLSLPVTPGEPASISCRSSQSLVHSNRNTYLHWYQQKPGQAPRLLIYKVSNRFSGVPDRFSGSGSGTDFTLKISRVEAEDVGVYYCSQNTHVPPTFGQGTKLEIKGGGGSQAVVTQESALTTSPGETVTLTCRSSTGAVTTSNYANWVQEKPDHLFTGLIGGTNKRAPGVPARFSGSLIGDKAALTITGAQTEDEAIYFCALWYSNLWVFGGGTKLTVLGGGGSGGGGSGGGGSEVKLLESGGGLVQPKGSLKLSCAASGFTFNTYAMNWVRQAPGKGLEWVARIRSKYNNYATYYADSVKDRFTISRDDSQSILYLQMNNLKTEDTAMYYCVRHGNFGNSYVSWFAYWGQGTLVTVSAHHHHHHHH

SEQ ID NO: 34 - protein, 753 aa, synthetic construct
  REGION 1..753: note = an artificially synthesized sequence
MGWSCIILFLVATATGVHSQVQLVQSGAEVKKPGASVKVSCKASGYTFTDYEMHWIRQPPGQGLEWIGAIDPKTGDTAYSQKFKGRVTLTADKSTSTAYMELSSLTSEDTAVYYCTRFYSYTYWGQGTLVTVSSGGGGSGGGGSGGGGSDIVMTQSPLSLPVTPGEPASISCRSSQSLVHSNRNTYLHWYQQKPGQAPRLLIYKVSNRFSGVPDRFSGSGSGTDFTLKISRVEAEDVGVYYCSQNTHVPPTFGQGTKLEIKGGGGSQAVVTQESALTTSPGETVTLTCRSSTGAVTTSNYANWVQEKPDHLFTGLIGGTNKRAPGVPARFSGSLIGDKAALTITGAQTEDEAIYFCALWYSNLWVFGGGTKLTVLGGGGSGGGGSGGGGSEVKLLESGGGLVQPKGSLKLSCAASGFTFNTYAMNWVRQAPGKGLEWVARIRSKYNNYATYYADSVKDRFTISRDDSQSILYLQMNNLKTEDTAMYYCVRHGNFGNSYVSWFAYWGQGTLVTVSAEPKSSDKTHTCPPCPAPEAAGGPSVFLFPPKPKDTLMISRTPEVTCVVVDVSHEDPEVKFNWYVDGVEVHNAKTKPREEQYASTYRVVSVLTVLHQDWLNGKEYKCKVSNKALPAPIEKTISKAKGQPREPQVCTLPPSRDELTKNQVSLWCLVKGFYPSDIAVEWESNGQPENNYKTTPPVLDSDGSFFLYSKLTVDKSRWQQGNVFSCSVMHEALHNHYTQKSLSLSPHHHHHHHH

SEQ ID NO: 35 - protein, 257 aa, synthetic construct
  REGION 1..257: note = an artificially synthesized sequence
MGWSCIILFLVATATGVHSEPKSSDKTHTCPPCPAPEAAGGPSVFLFPPKPKDTLMISRTPEVTCVVVDVSHEDPEVKFNWYVDGVEVHNAKTKPREEQYASTYRVVSVLTVLHQDWLNGKEYKCKVSNKALPAPIEKTISKAKGQPREPQVYTLPPSRCELTKNQVSLSCAVKGFYPSDIAVEWESNGQPENNYKTTPPVLDSDGSFFLVSKLTVDKSRWQQGNVFSCSVMHEALHNHYTQKSLSLSPDYKDDDDK

SEQ ID NO: 36 - protein, 514 aa, synthetic construct [sequence omitted]

SEQ ID NO: 37 - protein, 629 aa, synthetic construct
  REGION 1..629: note = an artificially synthesized sequence
MGWSCIILFLVATATGVHSQVQLVQSGAEVKKPGASVKVSCKASGYTFTDYEMHWIRQPPGQGLEWIGAIDPKTGDTAYSQKFKGRVTLTADKSTSTAYMELSSLTSEDTAVYYCTRFYSYTYWGQGTLVTVSSGGGGSGGGGSGGGGSDIVMTQSPLSLPVTPGEPASISCRSSQSLVHSNRNTYLHWYQQKPGQAPRLLIYKVSNRFSGVPDRFSGSGSGTDFTLKISRVEAEDVGVYYCSQNTHVPPTFGQGTKLEIKGGGGSEVKLLESGGGLVQPKGSLKLSCAASGFTFNTYAMNWVRQAPGKGLEWVARIRSKYNNYATYYADSVKDRFTISRDDSQSILYLQMNNLKTEDTAMYYCVRHGNFGNSYVSWFAYWGQGTLVTVSAEPKSSDKTHTCPPCPAPEAAGGPSVFLFPPKPKDTLMISRTPEVTCVVVDVSHEDPEVKFNWYVDGVEVHNAKTKPREEQYASTYRVVSVLTVLHQDWLNGKEYKCKVSNKALPAPIEKTISKAKGQPREPQVCTLPPSRDELTKNQVSLWCLVKGFYPSDIAVEWESNGQPENNYKTTPPVLDSDGSFFLYSKLTVDKSRWQQGNVFSCSVMHEALHNHYTQKSLSLSPHHHHHHHH

SEQ ID NO: 38 - protein, 613 aa, synthetic construct
  REGION 1..613: note = an artificially synthesized sequence
MGWSCIILFLVATATGVHSQVQLVQSGAEVKKPGASVKVSCKASGYTFTDYEMHWIRQPPGQGLEWIGAIDPKTGDTAYSQKFKGRVTLTADKSTSTAYMELSSLTSEDTAVYYCTRFYSYTYWGQGTLVTVSSGGGGSGGGGSGGGGSDIVMTQSPLSLPVTPGEPASISCRSSQSLVHSNRNTYLHWYQQKPGQAPRLLIYKVSNRFSGVPDRFSGSGSGTDFTLKISRVEAEDVGVYYCSQNTHVPPTFGQGTKLEIKGGGGSQAVVTQESALTTSPGETVTLTCRSSTGAVTTSNYANWVQEKPDHLFTGLIGGTNKRAPGVPARFSGSLIGDKAALTITGAQTEDEAIYFCALWYSNLWVFGGGTKLTVLEPKSSDKTHTCPPCPAPEAAGGPSVFLFPPKPKDTLMISRTPEVTCVVVDVSHEDPEVKFNWYVDGVEVHNAKTKPREEQYASTYRVVSVLTVLHQDWLNGKEYKCKVSNKALPAPIEKTISKAKGQPREPQVYTLPPSRCELTKNQVSLSCAVKGFYPSDIAVEWESNGQPENNYKTTPPVLDSDGSFFLVSKLTVDKSRWQQGNVFSCSVMHEALHNHYTQKSLSLSPDYKDDDDK

SEQ ID NO: 39 - protein, 470 aa, synthetic construct
  REGION 1..470: note = an artificially synthesized sequence
MGWSCIILFLVATATGVHSQVQLVQSGAEVKKPGASVKVSCKASGYTFTDYEMHWIRQPPGQGLEWIGAIDPKTGDTAYSQKFKGRVTLTADKSTSTAYMELSSLTSEDTAVYYCTRFYSYTYWGQGTLVTVSSASTKGPSVFPLAPSSKSTSGGTAALGCLVKDYFPEPVTVSWNSGALTSGVHTFPAVLQSSGLYSLSSVVTVPSSSLGTQTYICNVNHKPSNTKVDKKVEPKSCDKTHTCPPCPAPEAAGGPSVFLFPPKPKDTLMISRTPEVTCVVVDVSHEDPEVKFNWYVDGVEVHNAKTKPREEQYASTYRVVSVLTVLHQDWLNGKEYKCKVSNKALPAPIEKTISKAKGQPREPQVYTLPPSRCELTKNQVSLSCAVKGFYPSDIAVEWESNGQPENNYKTTPPVLDSDGSFFLVSKLTVDKSRWQQGNVFSCSVMHEALHNHYTQKSLSLSPDYKDDDDK

SEQ ID NO: 40 - protein, 238 aa, synthetic construct
  REGION 1..238: note = an artificially synthesized sequence
MGWSCIILFLVATATGVHSDIVMTQSPLSLPVTPGEPASISCRSSQSLVHSNRNTYLHWYQQKPGQAPRLLIYKVSNRFSGVPDRFSGSGSGTDFTLKISRVEAEDVGVYYCSQNTHVPPTFGQGTKLEIKRTVAAPSVFIFPPSDEQLKSGTASVVCLLNNFYPREAKVQWKVDNALQSGNSQESVTEQDSKDSTYSLSSTLTLSKADYEKHKVYACEVTHQGLSSPVTKSFNRGEC

SEQ ID NO: 41 - protein, 470 aa, synthetic construct
  REGION 1..470: note = an artificially synthesized sequence
MGWSCIILFLVATATGVHSQVQLVQSGAEVKKPGASVKVSCKASGYTFTDYEMHWIRQPPGQGLEWIGAIDPKTGDTAYSQKFKGRVTLTADKSTSTAYMELSSLTSEDTAVYYCTRFYSYTYWGQGTLVTVSSASTKGPSVFPLAPSSKSTSGGTAALGCLVKDYFPEPVTVSWNSGALTSGVHTFPAVLQSSGLYSLSSVVTVPSSSLGTQTYICNVNHKPSNTKVDKKVEPKSCDKTHTCPPCPAPEAAGGPSVFLFPPKPKDTLMISRTPEVTCVVVDVSHEDPEVKFNWYVDGVEVHNAKTKPREEQYASTYRVVSVLTVLHQDWLNGKEYKCKVSNKALPAPIEKTISKAKGQPREPQVCTLPPSRDELTKNQVSLWCLVKGFYPSDIAVEWESNGQPENNYKTTPPVLDSDGSFFLYSKLTVDKSRWQQGNVFSCSVMHEALHNHYTQKSLSLSPHHHHHHHH

SEQ ID NO: 42 - protein, 734 aa, synthetic construct [sequence omitted]

SEQ ID NO: 43 - protein, 462 aa, synthetic construct
  REGION 1..462: note = an artificially synthesized sequence
MGWSCIILFLVATATGVHSQVQLVQSGAEVKKPGASVKVSCKASGYTFTDYEMHWIRQPPGQGLEWIGAIDPKTGDTAYSQKFKGRVTLTADKSTSTAYMELSSLTSEDTAVYYCTRFYSYTYWGQGTLVTVSSASTKGPSVFPLAPSSKSTSGGTAALGCLVKDYFPEPVTVSWNSGALTSGVHTFPAVLQSSGLYSLSSVVTVPSSSLGTQTYICNVNHKPSNTKVDKKVEPKSCDKTHTCPPCPAPEAAGGPSVFLFPPKPKDTLMISRTPEVTCVVVDVSHEDPEVKFNWYVDGVEVHNAKTKPREEQYASTYRVVSVLTVLHQDWLNGKEYKCKVSNKALPAPIEKTISKAKGQPREPQVYTLPPSRDELTKNQVSLTCLVKGFYPSDIAVEWESNGQPENNYKTTPPVLDSDGSFFLYSKLTVDKSRWQQGNVFSCSVMHEALHNHYTQKSLSLSP

SEQ ID NO: 44 - protein, 246 aa, synthetic construct
  REGION 1..246: note = an artificially synthesized sequence
MGWSCIILFLVATATGVHSDIVMTQSPLSLPVTPGEPASISCRSSQSLVHSNRNTYLHWYQQKPGQAPRLLIYKVSNRFSGVPDRFSGSGSGTDFTLKISRVEAEDVGVYYCSQNTHVPPTFGQGTKLEIKRTVAAPSVFIFPPSDEQLKSGTASVVCLLNNFYPREAKVQWKVDNALQSGNSQESVTEQDSKDSTYSLSSTLTLSKADYEKHKVYACEVTHQGLSSPVTKSFNRGECHHHHHHHH

SEQ ID NO: 45 - protein, 505 aa, synthetic construct
  REGION 1..505: note = an artificially synthesized sequence
MGWSCIILFLVATATGVHSDIVMTQSPLSLPVTPGEPASISCRSSQSLVHSNRNTYLHWYQQKPGQAPRLLIYKVSNRFSGVPDRFSGSGSGTDFTLKISRVEAEDVGVYYCSQNTHVPPTFGQGTKLEIKRTVAAPSVFIFPPSDEQLKSGTASVVCLLNNFYPREAKVQWKVDNALQSGNSQESVTEQDSKDSTYSLSSTLTLSKADYEKHKVYACEVTHQGLSSPVTKSFNRGECGGGGSGGGGSQAVVTQESALTTSPGETVTLTCRSSTGAVTTSNYANWVQEKPDHLFTGLIGGTNKRAPGVPARFSGSLIGDKAALTITGAQTEDEAIYFCALWYSNLWVFGGGTKLTVLGGGGSGGGGSGGGGSEVKLLESGGGLVQPKGSLKLSCAASGFTFNTYAMNWVRQAPGKGLEWVARIRSKYNNYATYYADSVKDRFTISRDDSQSILYLQMNNLKTEDTAMYYCVRHGNFGNSYVSWFAYWGQGTLVTVSADYKDDDDK

SEQ ID NO: 46 - protein, 729 aa, synthetic construct
  REGION 1..729: note = an artificially synthesized sequence
MGWSCIILFLVATATGVHSQVQLVQSGAEVKKPGASVKVSCKASGYTFTDYEMHWIRQPPGQGLEWIGAIDPKTGDTAYSQKFKGRVTLTADKSTSTAYMELSSLTSEDTAVYYCTRFYSYTYWGQGTLVTVSSASTKGPSVFPLAPSSKSTSGGTAALGCLVKDYFPEPVTVSWNSGALTSGVHTFPAVLQSSGLYSLSSVVTVPSSSLGTQTYICNVNHKPSNTKVDKKVEPKSCDKTHTCPPCPAPEAAGGPSVFLFPPKPKDTLMISRTPEVTCVVVDVSHEDPEVKFNWYVDGVEVHNAKTKPREEQYASTYRVVSVLTVLHQDWLNGKEYKCKVSNKALPAPIEKTISKAKGQPREPQVYTLPPSRCELTKNQVSLSCAVKGFYPSDIAVEWESNGQPENNYKTTPPVLDSDGSFFLVSKLTVDKSRWQQGNVFSCSVMHEALHNHYTQKSLSLSPGGGGSGGGGSQAVVTQESALTTSPGETVTLTCRSSTGAVTTSNYANWVQEKPDHLFTGLIGGTNKRAPGVPARFSGSLIGDKAALTITGAQTEDEAIYFCALWYSNLWVFGGGTKLTVLGGGGSGGGGSGGGGSEVKLLESGGGLVQPKGSLKLSCAASGFTFNTYAMNWVRQAPGKGLEWVARIRSKYNNYATYYADSVKDRFTISRDDSQSILYLQMNNLKTEDTAMYYCVRHGNFGNSYVSWFAYWGQGTLVTVSADYKDDDDK

SEQ ID NO: 47 - protein, 729 aa, synthetic construct
  REGION 1..729: note = an artificially synthesized sequence
MGWSCIILFLVATATGVHSQVQLVQSGAEVKKPGASVKVSCKASGYTFTDYEMHWIRQPPGQGLEWIGAIDPKTGDTAYSQKFKGRVTLTADKSTSTAYMELSSLTSEDTAVYYCTRFYSYTYWGQGTLVTVSSASTKGPSVFPLAPSSKSTSGGTAALGCLVKDYFPEPVTVSWNSGALTSGVHTFPAVLQSSGLYSLSSVVTVPSSSLGTQTYICNVNHKPSNTKVDKKVEPKSCDKTHTCPPCPAPELLGGPSVFLFPPKPKDTLMISRTPEVTCVVVDVSHEDPEVKFNWYVDGVEVHNAKTKPREEQYNSTYRVVSVLTVLHQDWLNGKEYKCKVSNKALPAPIEKTISKAKGQPREPQVYTLPPSRCELTKNQVSLSCAVKGFYPSDIAVEWESNGQPENNYKTTPPVLDSDGSFFLVSKLTVDKSRWQQGNVFSCSVMHEALHNHYTQKSLSLSPGGGGSGGGGSQAVVTQESALTTSPGETVTLTCRSSTGAVTTSNYANWVQEKPDHLFTGLIGGTNKRAPGVPARFSGSLIGDKAALTITGAQTEDEAIYFCALWYSNLWVFGGGTKLTVLGGGGSGGGGSGGGGSEVKLLESGGGLVQPKGSLKLSCAASGFTFNTYAMNWVRQAPGKGLEWVARIRSKYNNYATYYADSVKDRFTISRDDSQSILYLQMNNLKTEDTAMYYCVRHGNFGNSYVSWFAYWGQGTLVTVSADYKDDDDK

SEQ ID NO: 48 - protein, 470 aa, synthetic construct
  REGION 1..470: note = an artificially synthesized sequence
MGWSCIILFLVATATGVHSQVQLVQSGAEVKKPGASVKVSCKASGYTFTDYEMHWIRQPPGQGLEWIGAIDPKTGDTAYSQKFKGRVTLTADKSTSTAYMELSSLTSEDTAVYYCTRFYSYTYWGQGTLVTVSSASTKGPSVFPLAPSSKSTSGGTAALGCLVKDYFPEPVTVSWNSGALTSGVHTFPAVLQSSGLYSLSSVVTVPSSSLGTQTYICNVNHKPSNTKVDKKVEPKSCDKTHTCPPCPAPELLGGPSVFLFPPKPKDTLMISRTPEVTCVVVDVSHEDPEVKFNWYVDGVEVHNAKTKPREEQYNSTYRVVSVLTVLHQDWLNGKEYKCKVSNKALPAPIEKTISKAKGQPREPQVCTLPPSRDELTKNQVSLWCLVKGFYPSDIAVEWESNGQPENNYKTTPPVLDSDGSFFLYSKLTVDKSRWQQGNVFSCSVMHEALHNHYTQKSLSLSPHHHHHHHH

SEQ ID NO: 49 - protein, 600 aa, synthetic construct
  REGION 1..600: note = an artificially synthesized sequence
MGWSCIILFLVATATGVHSQVQLVQSGAEVKKPGASVKVSCKASGYTFTDYEMHWIRQPPGQGLEWIGAIDPKTGDTAYSQKFKGRVTLTADKSTSTAYMELSSLTSEDTAVYYCTRFYSYTYWGQGTLVTVSSASTKGPSVFPLAPSSKSTSGGTAALGCLVKDYFPEPVTVSWNSGALTSGVHTFPAVLQSSGLYSLSSVVTVPSSSLGTQTYICNVNHKPSNTKVDKKVEPKSCDKTHTCPPCPAPEAAGGPSVFLFPPKPKDTLMISRTPEVTCVVVDVSHEDPEVKFNWYVDGVEVHNAKTKPREEQYASTYRVVSVLTVLHQDWLNGKEYKCKVSNKALPAPIEKTISKAKGQPREPQVYTLPPSRCELTKNQVSLSCAVKGFYPSDIAVEWESNGQPENNYKTTPPVLDSDGSFFLVSKLTVDKSRWQQGNVFSCSVMHEALHNHYTQKSLSLSPGGGGSEVKLLESGGGLVQPKGSLKLSCAASGFTFNTYAMNWVRQAPGKGLEWVARIRSKYNNYATYYADSVKDRFTISRDDSQSILYLQMNNLKTEDTAMYYCVRHGNFGNSYVSWFAYWGQGTLVTVSADYKDDDDK

SEQ ID NO: 50 - protein, 584 aa, synthetic construct
  REGION 1..584: note = an artificially synthesized sequence
MGWSCIILFLVATATGVHSQVQLVQSGAEVKKPGASVKVSCKASGYTFTDYEMHWIRQPPGQGLEWIGAIDPKTGDTAYSQKFKGRVTLTADKSTSTAYMELSSLTSEDTAVYYCTRFYSYTYWGQGTLVTVSSASTKGPSVFPLAPSSKSTSGGTAALGCLVKDYFPEPVTVSWNSGALTSGVHTFPAVLQSSGLYSLSSVVTVPSSSLGTQTYICNVNHKPSNTKVDKKVEPKSCDKTHTCPPCPAPEAAGGPSVFLFPPKPKDTLMISRTPEVTCVVVDVSHEDPEVKFNWYVDGVEVHNAKTKPREEQYASTYRVVSVLTVLHQDWLNGKEYKCKVSNKALPAPIEKTISKAKGQPREPQVCTLPPSRDELTKNQVSLWCLVKGFYPSDIAVEWESNGQPENNYKTTPPVLDSDGSFFLYSKLTVDKSRWQQGNVFSCSVMHEALHNHYTQKSLSLSPGGGGSQAVVTQESALTTSPGETVTLTCRSSTGAVTTSNYANWVQEKPDHLFTGLIGGTNKRAPGVPARFSGSLIGDKAALTITGAQTEDEAIYFCALWYSNLWVFGGGTKLTVLHHHHHHHH

SEQ ID NO: 51 - protein, 605 aa, synthetic construct
  REGION 1..605: note = an artificially synthesized sequence
MGWSCIILFLVATATGVHSQVQLVQSGAEVKKPGASVKVSCKASGYTFTDYEMHWIRQPPGQGLEWIGAIDPKTGDTAYSQKFKGRVTLTADKSTSTAYMELSSLTSEDTAVYYCTRFYSYTYWGQGTLVTVSSASTKGPSVFPLAPSSKSTSGGTAALGCLVKDYFPEPVTVSWNSGALTSGVHTFPAVLQSSGLYSLSSVVTVPSSSLGTQTYICNVNHKPSNTKVDKKVEPKSCDKTHTCPPCPAPEAAGGPSVFLFPPKPKDTLMISRTPEVTCVVVDVSHEDPEVKFNWYVDGVEVHNAKTKPREEQYASTYRVVSVLTVLHQDWLNGKEYKCKVSNKALPAPIEKTISKAKGQPREPQVYTLPPSRCELTKNQVSLSCAVKGFYPSDIAVEWESNGQPENNYKTTPPVLDSDGSFFLVSKLTVDKSRWQQGNVFSCSVMHEALHNHYTQKSLSLSPGGGGSGGGGSEVKLLESGGGLVQPKGSLKLSCAASGFTFNTYAMNWVRQAPGKGLEWVARIRSKYNNYATYYADSVKDRFTISRDDSQSILYLQMNNLKTEDTAMYYCVRHGNFGNSYVSWFAYWGQGTLVTVSADYKDDDDK

SEQ ID NO: 52 - protein, 589 aa, synthetic construct
  REGION 1..589: note = an artificially synthesized sequence
MGWSCIILFLVATATGVHSQVQLVQSGAEVKKPGASVKVSCKASGYTFTDYEMHWIRQPPGQGLEWIGAIDPKTGDTAYSQKFKGRVTLTADKSTSTAYMELSSLTSEDTAVYYCTRFYSYTYWGQGTLVTVSSASTKGPSVFPLAPSSKSTSGGTAALGCLVKDYFPEPVTVSWNSGALTSGVHTFPAVLQSSGLYSLSSVVTVPSSSLGTQTYICNVNHKPSNTKVDKKVEPKSCDKTHTCPPCPAPEAAGGPSVFLFPPKPKDTLMISRTPEVTCVVVDVSHEDPEVKFNWYVDGVEVHNAKTKPREEQYASTYRVVSVLTVLHQDWLNGKEYKCKVSNKALPAPIEKTISKAKGQPREPQVCTLPPSRDELTKNQVSLWCLVKGFYPSDIAVEWESNGQPENNYKTTPPVLDSDGSFFLYSKLTVDKSRWQQGNVFSCSVMHEALHNHYTQKSLSLSPGGGGSGGGGSQAVVTQESALTTSPGETVTLTCRSSTGAVTTSNYANWVQEKPDHLFTGLIGGTNKRAPGVPARFSGSLIGDKAALTITGAQTEDEAIYFCALWYSNLWVFGGGTKLTVLHHHHHHHH

SEQ ID NO: 53 - protein, 610 aa, synthetic construct
  REGION 1..610: note = an artificially synthesized sequence
MGWSCIILFLVATATGVHSQVQLVQSGAEVKKPGASVKVSCKASGYTFTDYEMHWIRQPPGQGLEWIGAIDPKTGDTAYSQKFKGRVTLTADKSTSTAYMELSSLTSEDTAVYYCTRFYSYTYWGQGTLVTVSSASTKGPSVFPLAPSSKSTSGGTAALGCLVKDYFPEPVTVSWNSGALTSGVHTFPAVLQSSGLYSLSSVVTVPSSSLGTQTYICNVNHKPSNTKVDKKVEPKSCDKTHTCPPCPAPEAAGGPSVFLFPPKPKDTLMISRTPEVTCVVVDVSHEDPEVKFNWYVDGVEVHNAKTKPREEQYASTYRVVSVLTVLHQDWLNGKEYKCKVSNKALPAPIEKTISKAKGQPREPQVYTLPPSRCELTKNQVSLSCAVKGFYPSDIAVEWESNGQPENNYKTTPPVLDSDGSFFLVSKLTVDKSRWQQGNVFSCSVMHEALHNHYTQKSLSLSPGGGGSGGGGSGGGGSEVKLLESGGGLVQPKGSLKLSCAASGFTFNTYAMNWVRQAPGKGLEWVARIRSKYNNYATYYADSVKDRFTISRDDSQSILYLQMNNLKTEDTAMYYCVRHGNFGNSYVSWFAYWGQGTLVTVSADYKDDDDK

SEQ ID NO: 54 - protein, 594 aa, synthetic construct
  REGION 1..594: note = an artificially synthesized sequence
MGWSCIILFLVATATGVHSQVQLVQSGAEVKKPGASVKVSCKASGYTFTDYEMHWIRQPPGQGLEWIGAIDPKTGDTAYSQKFKGRVTLTADKSTSTAYMELSSLTSEDTAVYYCTRFYSYTYWGQGTLVTVSSASTKGPSVFPLAPSSKSTSGGTAALGCLVKDYFPEPVTVSWNSGALTSGVHTFPAVLQSSGLYSLSSVVTVPSSSLGTQTYICNVNHKPSNTKVDKKVEPKSCDKTHTCPPCPAPEAAGGPSVFLFPPKPKDTLMISRTPEVTCVVVDVSHEDPEVKFNWYVDGVEVHNAKTKPREEQYASTYRVVSVLTVLHQDWLNGKEYKCKVSNKALPAPIEKTISKAKGQPREPQVCTLPPSRDELTKNQVSLWCLVKGFYPSDIAVEWESNGQPENNYKTTPPVLDSDGSFFLYSKLTVDKSRWQQGNVFSCSVMHEALHNHYTQKSLSLSPGGGGSGGGGSGGGGSQAVVTQESALTTSPGETVTLTCRSSTGAVTTSNYANWVQEKPDHLFTGLIGGTNKRAPGVPARFSGSLIGDKAALTITGAQTEDEAIYFCALWYSNLWVFGGGTKLTVLHHHHHHHH

SEQ ID NO: 55 - protein, 615 aa, synthetic construct
  REGION 1..615: note = an artificially synthesized sequence
MGWSCIILFLVATATGVHSQVQLVQSGAEVKKPGASVKVSCKASGYTFTDYEMHWIRQPPGQGLEWIGAIDPKTGDTAYSQKFKGRVTLTADKSTSTAYMELSSLTSEDTAVYYCTRFYSYTYWGQGTLVTVSSASTKGPSVFPLAPSSKSTSGGTAALGCLVKDYFPEPVTVSWNSGALTSGVHTFPAVLQSSGLYSLSSVVTVPSSSLGTQTYICNVNHKPSNTKVDKKVEPKSCDKTHTCPPCPAPEAAGGPSVFLFPPKPKDTLMISRTPEVTCVVVDVSHEDPEVKFNWYVDGVEVHNAKTKPREEQYASTYRVVSVLTVLHQDWLNGKEYKCKVSNKALPAPIEKTISKAKGQPREPQVYTLPPSRCELTKNQVSLSCAVKGFYPSDIAVEWESNGQPENNYKTTPPVLDSDGSFFLVSKLTVDKSRWQQGNVFSCSVMHEALHNHYTQKSLSLSPGGGGSGGGGSGGGGSGGGGSEVKLLESGGGLVQPKGSLKLSCAASGFTFNTYAMNWVRQAPGKGLEWVARIRSKYNNYATYYADSVKDRFTISRDDSQSILYLQMNNLKTEDTAMYYCVRHGNFGNSYVSWFAYWGQGTLVTVSADYKDDDDK

SEQ ID NO: 56 - protein, 599 aa, synthetic construct
  REGION 1..599: note = an artificially synthesized sequence
MGWSCIILFLVATATGVHSQVQLVQSGAEVKKPGASVKVSCKASGYTFTDYEMHWIRQPPGQGLEWIGAIDPKTGDTAYSQKFKGRVTLTADKSTSTAYMELSSLTSEDTAVYYCTRFYSYTYWGQGTLVTVSSASTKGPSVFPLAPSSKSTSGGTAALGCLVKDYFPEPVTVSWNSGALTSGVHTFPAVLQSSGLYSLSSVVTVPSSSLGTQTYICNVNHKPSNTKVDKKVEPKSCDKTHTCPPCPAPEAAGGPSVFLFPPKPKDTLMISRTPEVTCVVVDVSHEDPEVKFNWYVDGVEVHNAKTKPREEQYASTYRVVSVLTVLHQDWLNGKEYKCKVSNKALPAPIEKTISKAKGQPREPQVCTLPPSRDELTKNQVSLWCLVKGFYPSDIAVEWESNGQPENNYKTTPPVLDSDGSFFLYSKLTVDKSRWQQGNVFSCSVMHEALHNHYTQKSLSLSPGGGGSGGGGSGGGGSGGGGSQAVVTQESALTTSPGETVTLTCRSSTGAVTTSNYANWVQEKPDHLFTGLIGGTNKRAPGVPARFSGSLIGDKAALTITGAQTEDEAIYFCALWYSNLWVFGGGTKLTVLHHHHHHHH

SEQ ID NO: 57 - protein, 610 aa, synthetic construct
  REGION 1..610: note = an artificially synthesized sequence
MGWSCIILFLVATATGVHSQVQLVQSGAEVKKPGASVKVSCKASGYTFTDYEMHWIRQPPGQGLEWIGAIDPKTGDTAYSQKFKGRVTLTADKSTSTAYMELSSLTSEDTAVYYCTRFYSYTYWGQGTLVTVSSASTKGPSVFPLAPSSKSTSGGTAALGCLVKDYFPEPVTVSWNSGALTSGVHTFPAVLQSSGLYSLSSVVTVPSSSLGTQTYICNVNHKPSNTKVDKKVEPKSCDKTHTCPPCPAPEAAGGPSVFLFPPKPKDTLMISRTPEVTCVVVDVSHEDPEVKFNWYVDGVEVHNAKTKPREEQYASTYRVVSVLTVLHQDWLNGKEYKCKVSNKALPAPIEKTISKAKGQPREPQVYTLPPSRCELTKNQVSLSCAVKGFYPSDIAVEWESNGQPENNYKTTPPVLDSDGSFFLVSKLTVDKSRWQQGNVFSCSVMHEALHNHYTQKSLSLSPGGGGSGGGGSGGGGSEVKLLESGGGLVQPKGSLKLSCAASGFTFNTYAMNWVRQAPGKCLEWVARIRSKYNNYATYYADSVKDRFTISRDDSQSILYLQMNNLKTEDTAMYYCVRHGNFGNSYVSWFAYWGQGTLVTVSADYKDDDDK

SEQ ID NO: 58 - protein, 594 aa, synthetic construct
  REGION 1..594: note = an artificially synthesized sequence
MGWSCIILFLVATATGVHSQVQLVQSGAEVKKPGASVKVSCKASGYTFTDYEMHWIRQPPGQGLEWIGAIDPKTGDTAYSQKFKGRVTLTADKSTSTAYMELSSLTSEDTAVYYCTRFYSYTYWGQGTLVTVSSASTKGPSVFPLAPSSKSTSGGTAALGCLVKDYFPEPVTVSWNSGALTSGVHTFPAVLQSSGLYSLSSVVTVPSSSLGTQTYICNVNHKPSNTKVDKKVEPKSCDKTHTCPPCPAPEAAGGPSVFLFPPKPKDTLMISRTPEVTCVVVDVSHEDPEVKFNWYVDGVEVHNAKTKPREEQYASTYRVVSVLTVLHQDWLNGKEYKCKVSNKALPAPIEKTISKAKGQPREPQVCTLPPSRDELTKNQVSLWCLVKGFYPSDIAVEWESNGQPENNYKTTPPVLDSDGSFFLYSKLTVDKSRWQQGNVFSCSVMHEALHNHYTQKSLSLSPGGGGSGGGGSGGGGSQAVVTQESALTTSPGETVTLTCRSSTGAVTTSNYANWVQEKPDHLFTGLIGGTNKRAPGVPARFSGSLIGDKAALTITGAQTEDEAIYFCALWYSNLWVFGCGTKLTVLHHHHHHHH

SEQ ID NO: 59 - protein, 704 aa, synthetic construct
  REGION 1..704: note = an artificially synthesized sequence
MGWSCIILFLVATATGVHSQVQLVQSGAEVKKPGASVKVSCKASGYTFTDYEMHWIRQPPGQGLEWIGAIDPKTGDTAYSQKFKGRVTLTADKSTSTAYMELSSLTSEDTAVYYCTRFYSYTYWGQGTLVTVSSASTKGPSVFPLAPSSKSTSGGTAALGCLVKDYFPEPVTVSWNSGALTSGVHTFPAVLQSSGLYSLSSVVTVPSSSLGTQTYICNVNHKPSNTKVDKKVEPKSCDKTHTCPPCPAPEAAGGPSVFLFPPKPKDTLMISRTPEVTCVVVDVSHEDPEVKFNWYVDGVEVHNAKTKPREEQYASTYRVVSVLTVLHQDWLNGKEYKCKVSNKALPAPIEKTISKAKGQPREPQVYTLPPSRCELTKNQVSLSCAVKGFYPSDIAVEWESNGQPENNYKTTPPVLDSDGSFFLVSKLTVDKSRWQQGNVFSCSVMHEALHNHYTQKSLSLSPGGGGSGGGGSGGGGSEVKLLESGGGLVQPKGSLKLSCAASGFTFNTYAMNWVRQAPGKGLEWVARIRSKYNNYATYYADSVKDRFTISRDDSQSILYLQMNNLKTEDTAMYYCVRHGNFGNSYVSWFAYWGQGTLVTVSAASTKGPSVFPLAPSSKSTSGGTAALGCLVKDYFPEPVTVSWNSGALTSGVHTFPAVLQSSGLYSLSSVVTVPSSSLGTQTYICNVNHKPSNTKVDKKVEPKS

SEQ ID NO: 60 - protein, 692 aa, synthetic construct [sequence omitted]

SEQ ID NO: 61 - protein, 115 aa, synthetic construct
  REGION 1..115: note = an artificially synthesized sequence
QVQLVQSGAEVKKPGASVKVSCKASGYTFTDYEMHWIRQPPGQGLEWIGAIDPKTGDTAYSQKFKGRVTLTADKSTSTAYMELSSLTSEDTAVYYCTRFYSYTYWGQGTLVTVSS

SEQ ID NO: 62 - protein, 219 aa, synthetic construct
  REGION 1..219: note = an artificially synthesized sequence
DVVMTQSPLSLPVTPGEPASISCRSSQSLVHSNRNTYLHWYLQKPGQSPQLLIYKVSNRFSGVPDRFSGSGSGTDFTLKISRVEAEDVGVYYCSQNTHVPPTFGQGTKLEIKRTVAAPSVFIFPPSDEQLKSGTASVVCLLNNFYPREAKVQWKVDNALQSGNSQESVTEQDSKDSTYSLSSTLTLSKADYEKHKVYACEVTHQGLSSPVTKSFNRGEC

SEQ ID NO: 63 - protein, 328 aa, synthetic construct
  REGION 1..328: note = an artificially synthesized sequence
ASTKGPSVFPLAPSSKSTSGGTAALGCLVKDYFPEPVTVSWNSGALTSGVHTFPAVLQSSGLYSLSSVVTVPSSSLGTQTYICNVNHKPSNTKVDKKVEPKSCDKTHTCPPCPAPEAAGGPSVFLFPPKPKDTLMISRTPEVTCVVVDVSHEDPEVKFNWYVDGVEVHNAKTKPREEQYASTYRVVSVLTVLHQDWLNGKEYKCKVSNKALPAPIEKTISKAKGQPREPQVYTLPPSRDELTKNQVSLTCLVKGFYPSDIAVEWESNGQPENNYKTTPPVLDSDGSFFLYSKLTVDKSRWQQGNVFSCSVMHEALHNHYTQKSLSLSP

SEQ ID NO: 64 - protein, 587 aa, synthetic construct
  REGION 1..587: note = an artificially synthesized sequence
ASTKGPSVFPLAPSSKSTSGGTAALGCLVKDYFPEPVTVSWNSGALTSGVHTFPAVLQSSGLYSLSSVVTVPSSSLGTQTYICNVNHKPSNTKVDKKVEPKSCDKTHTCPPCPAPEAAGGPSVFLFPPKPKDTLMISRTPEVTCVVVDVSHEDPEVKFNWYVDGVEVHNAKTKPREEQYASTYRVVSVLTVLHQDWLNGKEYKCKVSNKALPAPIEKTISKAKGQPREPQVYTLPPSRDELTKNQVSLTCLVKGFYPSDIAVEWESNGQPENNYKTTPPVLDSDGSFFLYSKLTVDKSRWQQGNVFSCSVMHEALHNHYTQKSLSLSPGGGGSGGGGSQAVVTQESALTTSPGETVTLTCRSSTGAVTTSNYANWVQEKPDHLFTGLIGGTNKRAPGVPARFSGSLIGDKAALTITGAQTEDEAIYFCALWYSNLWVFGGGTKLTVLGGGGSGGGGSGGGGSEVKLLESGGGLVQPKGSLKLSCAASGFTFNTYAMNWVRQAPGKGLEWVARIRSKYNNYATYYADSVKDRFTISRDDSQSILYLQMNNLKTEDTAMYYCVRHGNFGNSYVSWFAYWGQGTLVTVSA

SEQ ID NO: 65 - protein, 328 aa, synthetic construct
  REGION 1..328: note = an artificially synthesized sequence
ASTKGPSVFPLAPSSKSTSGGTAALGCLVKDYFPEPVTVSWNSGALTSGVHTFPAVLQSSGLYSLSSVVTVPSSSLGTQTYICNVNHKPSNTKVDKKVEPKSCDKTHTCPPCPAPEAAGGPSVFLFPPKPKDTLMISRTPEVTCVVVDVSHEDPEVKFNWYVDGVEVHNAKTKPREEQYASTYRVVSVLTVLHQDWLNGKEYKCKVSNKALPAPIEKTISKAKGQPREPQVYTLPPSRDELTKNQVSLTCLVKGFYPSDIAVEWESNGQPENNYKTTPPVLDSDGSFFLYSKLTVDKSRWQQGNVFSCSVMHEALHNRYTQESLSLSP

SEQ ID NO: 66 - protein, 587 aa, synthetic construct
  REGION 1..587: note = an artificially synthesized sequence
ASTKGPSVFPLAPSSKSTSGGTAALGCLVKDYFPEPVTVSWNSGALTSGVHTFPAVLQSSGLYSLSSVVTVPSSSLGTQTYICNVNHKPSNTKVDKKVEPKSCDKTHTCPPCPAPEAAGGPSVFLFPPKPKDTLMISRTPEVTCVVVDVSHEDPEVKFNWYVDGVEVHNAKTKPREEQYASTYRVVSVLTVLHQDWLNGKEYKCKVSNKALPAPIEKTISKAKGQPREPQVYTLPPSRKELTKNQVSLTCLVKGFYPSDIAVEWESNGQPENNYKTTPPVLDSDGSFFLYSKLTVDKSRWQQGNVFSCSVMHEALHNHYTQKSLSLSPGGGGSGGGGSQAVVTQESALTTSPGETVTLTCRSSTGAVTTSNYANWVQEKPDHLFTGLIGGTNKRAPGVPARFSGSLIGDKAALTITGAQTEDEAIYFCALWYSNLWVFGGGTKLTVLGGGGSGGGGSGGGGSEVKLLESGGGLVQPKGSLKLSCAASGFTFNTYAMNWVRQAPGKGLEWVARIRSKYNNYATYYADSVKDRFTISRDDSQSILYLQMNNLKTEDTAMYYCVRHGNFGNSYVSWFAYWGQGTLVTVSA

SEQ ID NO: 67 - protein, 141 aa, Homo sapiens
DIQNPDPAVYQLRDSKSSDKSVCLFTDFDSQTNVSQSKDSDVYITDKTVLDMRSMDFKSNSAVAWSNKSDFACANAFNNSIIPEDTFFPSPESSCDVKLVEKSFETDTNLNFQNLSVIGFRILLLKVAGFNLLMTLRLWSS

SEQ ID NO: 68 - protein, 179 aa, Homo sapiens
EDLKNVFPPEVAVFEPSEAEISHTQKATLVCLATGFYPDHVELSWWVNGKEVHSGVSTDPQPLKEQPALNDSRYCLSSRLRVSATFWQNPRNHFRCQVQFYGLSENDEWTQDRAKPVTQIVSAEAWGRADCGFTSESYQQGVLSATILYEILLGKATLYAVLVSALVLMAMVKRKDSRG

SEQ ID NO: 69 - protein, 173 aa, Homo sapiens
DKQLDADVSPKPTIFLPSIAETKLQKAGTYLCLLEKFFPDVIKIHWQEKKSNTILGSQEGNTMKTNDTYMKFSWLTVPEKSLDKEHRCIVRHENNKNGVDQEIIFPPIKTDVITMDPKDNCSKDANDTLLLQLTNTSAYYMYLLLLLKSVVYFAIITCCLLRRTAFCCNGEKS

SEQ ID NO: 70 - protein, 204 aa, Homo sapiens
KQLDADVSPKPTIFLPSIAETKLQKAGTYLCLLEKFFPDIIKIHWQEKKSNTILGSQEGNTMKTNDTYMKFSWLTVPEESLDKEHRCIVRHENNKNGIDQEIIFPPIKTDVTTVDPKDSYSKDANDVTTVDPKYNYSKDANDVITMDPKDNWSKDANDTLLLQLTNTSAYYMYLLLLLKSVVYFAIITCCLLGRTAFCCNGEKS

SEQ ID NO: 71 - protein, 177 aa, Homo sapiens
PSYTGGYADKLIFGKGTRVTVEPRSQPHTKPSVFVMKNGTNVACLVKEFYPKDIRINLVSSKKITEFDPAIVISPSGKYNAVKLGKYEDSNSVTCSVQHDNKTVHSTDFEVKTDSTDHVKPKETENTKQPSKSCHKPKAIVHTEKVNMMSLTVLGLRMLFAKTVAVNFLLTAKLFFL

SEQ ID NO: 72 - protein, 19 aa, synthetic construct
  REGION 1..19: note = signal sequence
MGWSCIILFLVATATGVHS

SEQ ID NO: 73 - protein, 466 aa, synthetic construct
  REGION 1..466: note = an artificially synthesized sequence
MGWSCIILFLVATATGVHSQAVVTQESALTTSPGETVTLTCRSSTGAVTTSNYANWVQEKPDHLFTGLIGGTNKRAPGVPARFSGSLIGDKAALTITGAQTEDEAIYFCALWYSNLWVFGGGTKLTVLSSASTKGPSVFPLAPSSKSTSGGTAALGCLVKDYFPEPVTVSWNSGALTSGVHTFPAVLQSSGLYSLSSVVTVPSSSLGTQTYICNVNHKPSNTKVDKKVEPKSCDKTHTCPPCPAPEAAGGPSVFLFPPKPKDTLMISRTPEVTCVVVDVSHEDPEVKFNWYVDGVEVHNAKTKPREEQYASTYRVVSVLTVLHQDWLNGKEYKCKVSNKALPAPIEKTISKAKGQPREPQVYTLPPSRCELTKNQVSLSCAVKGFYPSDIAVEWESNGQPENNYKTTPPVLDSDGSFFLVSKLTVDKSRWQQGNVFSCSVMHEALHNHYTQKSLSLSPDYKDDDDK

SEQ ID NO: 74 - protein, 251 aa, synthetic construct
  REGION 1..251: note = an artificially synthesized sequence
MGWSCIILFLVATATGVHSEVKLLESGGGLVQPKGSLKLSCAASGFTFNTYAMNWVRQAPGKGLEWVARIRSKYNNYATYYADSVKDRFTISRDDSQSILYLQMNNLKTEDTAMYYCVRHGNFGNSYVSWFAYWGQGTLVTVSAASVAAPSVFIFPPSDEQLKSGTASVVCLLNNFYPREAKVQWKVDNALQSGNSQESVTEQDSKDSTYSLSSTLTLSKADYEKHKVYACEVTHQGLSSPVTKSFNRGEC

SEQ ID NO: 75 - protein, 484 aa, synthetic construct
  REGION 1..484: note = an artificially synthesized sequence
MGWSCIILFLVATATGVHSEVKLLESGGGLVQPKGSLKLSCAASGFTFNTYAMNWVRQAPGKGLEWVARIRSKYNNYATYYADSVKDRFTISRDDSQSILYLQMNNLKTEDTAMYYCVRHGNFGNSYVSWFAYWGQGTLVTVSAASVAAPSVFIFPPSDEQLKSGTASVVCLLNNFYPREAKVQWKVDNALQSGNSQESVTEQDSKDSTYSLSSTLTLSKADYEKHKVYACEVTHQGLSSPVTKSFNRGECDKTHTCPPCPAPEAAGGPSVFLFPPKPKDTLMISRTPEVTCVVVDVSHEDPEVKFNWYVDGVEVHNAKTKPREEQYASTYRVVSVLTVLHQDWLNGKEYKCKVSNKALPAPIEKTISKAKGQPREPQVYTLPPSRCELTKNQVSLSCAVKGFYPSDIAVEWESNGQPENNYKTTPPVLDSDGSFFLVSKLTVDKSRWQQGNVFSCSVMHEALHNHYTQKSLSLSPDYKDDDDK

SEQ ID NO: 76 - protein, 233 aa, synthetic construct
  REGION 1..233: note = an artificially synthesized sequence
MGWSCIILFLVATATGVHSQAVVTQESALTTSPGETVTLTCRSSTGAVTTSNYANWVQEKPDHLFTGLIGGTNKRAPGVPARFSGSLIGDKAALTITGAQTEDEAIYFCALWYSNLWVFGGGTKLTVLSSASTKGPSVFPLAPSSKSTSGGTAALGCLVKDYFPEPVTVSWNSGALTSGVHTFPAVLQSSGLYSLSSVVTVPSSSLGTQTYICNVNHKPSNTKVDKKVEPKSC

SEQ ID NO: 77 - protein, 466 aa, synthetic construct
  REGION 1..466: note = an artificially synthesized sequence
MGWSCIILFLVATATGVHSQTVVTQEPSLTVSPGGTVTLTCGSSTGAVTSGNYPNWVQQKPGQAPRGLIGGTKFLAPGTPARFSGSLLGGKAALTLSGVQPEDEAEYYCVLWYSNRWVFGGGTKLTVLSSASTKGPSVFPLAPSSKSTSGGTAALGCLVKDYFPEPVTVSWNSGALTSGVHTFPAVLQSSGLYSLSSVVTVPSSSLGTQTYICNVNHKPSNTKVDKKVEPKSCDKTHTCPPCPAPEAAGGPSVFLFPPKPKDTLMISRTPEVTCVVVDVSHEDPEVKFNWYVDGVEVHNAKTKPREEQYASTYRVVSVLTVLHQDWLNGKEYKCKVSNKALPAPIEKTISKAKGQPREPQVYTLPPSRCELTKNQVSLSCAVKGFYPSDIAVEWESNGQPENNYKTTPPVLDSDGSFFLVSKLTVDKSRWQQGNVFSCSVMHEALHNHYTQKSLSLSPDYKDDDDK

SEQ ID NO: 78 - protein, 251 aa, synthetic construct
  REGION 1..251: note = an artificially synthesized sequence
MGWSCIILFLVATATGVHSEVQLVESGGGLVQPGGSLKLSCAASGFTFNKYAMNWVRQAPGKGLEWVARIRSKYNNYATYYADSVKDRFTISRDDSKNTAYLQMNNLKTEDTAVYYCVRHGNFGNSYISYWAYWGQGTLVTVSSASVAAPSVFIFPPSDEQLKSGTASVVCLLNNFYPREAKVQWKVDNALQSGNSQESVTEQDSKDSTYSLSSTLTLSKADYEKHKVYACEVTHQGLSSPVTKSFNRGEC

SEQ ID NO: 79 - protein, 475 aa, synthetic construct
  REGION 1..475: note = an artificially synthesized sequence
MGWSCIILFLVATATGVHSEVQLLEQSGAELVRPGTSVKISCKASGYAFTNYWLGWVKQRPGHGLEWIGDIFPGSGNIHYNEKFKGKATLTADKSSSTAYMQLSSLTFEDSAVYFCARLRNWDEPMDYWGQGTTVTVSSASTKGPSVFPLAPSSKSTSGGTAALGCLVKDYFPEPVTVSWNSGALTSGVHTFPAVLQSSGLYSLSSVVTVPSSSLGTQTYICNVNHKPSNTKVDKKVEPKSCDKTHTCPPCPAPEAAGGPSVFLFPPKPKDTLMISRTPEVTCVVVDVSHEDPEVKFNWYVDGVEVHNAKTKPREEQYASTYRVVSVLTVLHQDWLNGKEYKCKVSNKALPAPIEKTISKAKGQPREPQVCTLPPSRDELTKNQVSLWCLVKGFYPSDIAVEWESNGQPENNYKTTPPVLDSDGSFFLYSKLTVDKSRWQQGNVFSCSVMHEALHNHYTQKSLSLSPHHHHHHHH

SEQ ID NO: 80 - protein, 239 aa, synthetic construct
  REGION 1..239: note = an artificially synthesized sequence
MGWSCIILFLVATATGVHSELVMTQSPSSLTVTAGEKVTMSCKSSQSLLNSGNQKNYLTWYQQKPGQPPKLLIYWASTRESGVPDRFTGSGSGTDFTLTISSVQAEDLAVYYCQNDYSYPLTFGAGTKLEIKRTVAAPSVFIFPPSDEQLKSGTASVVCLLNNFYPREAKVQWKVDNALQSGNSQESVTEQDSKDSTYSLSSTLTLSKADYEKHKVYACEVTHQGLSSPVTKSFNRGEC

SEQ ID NO: 81 - protein, 453 aa, synthetic construct
  REGION 1..453: note = an artificially synthesized sequence
EVKLLESGGGLVQPKGSLKLSCAASGFTFNTYAMNWVRQAPGKGLEWVARIRSKYNNYATYYADSVKDRFTISRDDSQSILYLQMNNLKTEDTAMYYCVRHGNFGNSYVSWFAYWGQGTLVTVSAASTKGPSVFPLAPSSKSTSGGTAALGCLVKDYFPEPVTVSWNSGALTSGVHTFPAVLQSSGLYSLSSVVTVPSSSLGTQTYICNVNHKPSNTKVDKKVEPKSCDKTHTCPPCPAPEAAGGPSVFLFPPKPKDTLMISRTPEVTCVVVDVSHEDPEVKFNWYVDGVEVHNAKTKPREEQYASTYRVVSVLTVLHQDWLNGKEYKCKVSNKALPAPIEKTISKAKGQPREPQVYTLPPSRDELTKNQVSLTCLVKGFYPSDIAVEWESNGQPENNYKTTPPVLDSDGSFFLYSKLTVDKSRWQQGNVFSCSVMHEALHNHYTQKSLSLSP

SEQ ID NO: 82 - protein, 216 aa, synthetic construct
  REGION 1..216: note = an artificially synthesized sequence
QAVVTQESALTTSPGETVTLTCRSSTGAVTTSNYANWVQEKPDHLFTGLIGGTNKRAPGVPARFSGSLIGDKAALTITGAQTEDEAIYFCALWYSNLWVFGGGTKLTVLRTVAAPSVFIFPPSDEQLKSGTASVVCLLNNFYPREAKVQWKVDNALQSGNSQESVTEQDSKDSTYSLSSTLTLSKADYEKHKVYACEVTHQGLSSPVTKSFNRGEC

SEQ ID NO: 83 - protein, 443 aa, synthetic construct
  REGION 1..443: note = an artificially synthesized sequence
QVQLVQSGAEVKKPGASVKVSCKASGYTFTDYEMHWIRQPPGQGLEWIGAIDPKTGDTAYSQKFKGRVTLTADKSTSTAYMELSSLTSEDTAVYYCTRFYSYTYWGQGTLVTVSSASTKGPSVFPLAPSSKSTSGGTAALGCLVKDYFPEPVTVSWNSGALTSGVHTFPAVLQSSGLYSLSSVVTVPSSSLGTQTYICNVNHKPSNTKVDKKVEPKSCDKTHTCPPCPAPEAAGGPSVFLFPPKPKDTLMISRTPEVTCVVVDVSHEDPEVKFNWYVDGVEVHNAKTKPREEQYASTYRVVSVLTVLHQDWLNGKEYKCKVSNKALPAPIEKTISKAKGQPREPQVYTLPPSRDELTKNQVSLTCLVKGFYPSDIAVEWESNGQPENNYKTTPPVLDSDGSFFLYSKLTVDKSRWQQGNVFSCSVMHEALHNHYTQKSLSLSP

SEQ ID NO: 84 - protein, 219 aa, synthetic construct
  REGION 1..219: note = an artificially synthesized sequence
DIVMTQSPLSLPVTPGEPASISCRSSQSLVHSNRNTYLHWYQQKPGQAPRLLIYKVSNRFSGVPDRFSGSGSGTDFTLKISRVEAEDVGVYYCSQNTHVPPTFGQGTKLEIKRTVAAPSVFIFPPSDEQLKSGTASVVCLLNNFYPREAKVQWKVDNALQSGNSQESVTEQDSKDSTYSLSSTLTLSKADYEKHKVYACEVTHQGLSSPVTKSFNRGEC

SEQ ID NO: 85 - protein, 453 aa, synthetic construct
  REGION 1..453: note = an artificially synthesized sequence
EVKLLESGGGLVQPKGSLKLSCAASGFTFNTYAMNWVRQAPGKGLEWVARIRSKYNNYATYYADSVKDRFTISRDDSQSILYLQMNNLKTEDTAMYYCVRHGNFGNSYVSWFAYWGQGTLVTVSAASTKGPSVFPLAPSSKSTSGGTAALGCLVKDYFPEPVTVSWNSGALTSGVHTFPAVLKSSGLYSLSSVVTVPSSSLGTQTYICNVNHKPSNTKVDKKVEPKSCDKTHTCPPCPAPEAAGGPSVFLFPPKPKDTLMISRTPEVTCVVVDVSHEDPEVKFNWYVDGVEVHNAKTKPREEQYASTYRVVSVLTVLHQDWLNGKEYKCKVSNKALPAPIEKTISKAKGQPREPQVYTLPPSRCELTKNQVSLSCAVKGFYPSDIAVEWESNGQPENNYKTTPPVLDSDGSFFLVSKLTVDKSRWQQGNVFSCSVMHEALHNHYTQKSLSLSP

SEQ ID NO: 86 - protein, 216 aa, synthetic construct
  REGION 1..216: note = an artificially synthesized sequence
QAVVTQESALTTSPGETVTLTCRSSTGAVTTSNYANWVQEKPDHLFTGLIGGTNKRAPGVPARFSGSLIGDKAALTITGAQTEDEAIYFCALWYSNLWVFGGGTKLTVLRTVAAPSVFIFPPSDEQLKSGTAEVVCLLNNFYPREAKVQWKVDNALQSGNSEESVTEQDSKDSTYSLSSTLELSKADYEKHKVYACEVTHQGLSSPVTKSFNRGEC

SEQ ID NO: 87 - protein, 443 aa, synthetic construct
  REGION 1..443: note = an artificially synthesized sequence
QVQLVQSGAEVKKPGASVKVSCKASGYTFTDYEMHWIRQPPGQGLEWIGAIDPKTGDTAYSQKFKGRVTLTADKSTSTAYMELSSLTSEDTAVYYCTRFYSYTYWGQGTLVTVSSASTKGPSVFPLAPSSKSTSGGTAALGCLVEDYFPEPVTVSWNSGALTSGVHTFPAVLESSGLYSLSSVVTVPSSSLGTQTYICNVNHKPSNTKVDKKVEPKSCDKTHTCPPCPAPEAAGGPSVFLFPPKPKDTLMISRTPEVTCVVVDVSHEDPEVKFNWYVDGVEVHNAKTKPREEQYASTYRVVSVLTVLHQDWLNGKEYKCKVSNKALPAPIEKTISKAKGQPREPQVCTLPPSRDELTKNQVSLWCLVKGFYPSDIAVEWESNGQPENNYKTTPPVLDSDGSFFLYSKLTVDKSRWQQGNVFSCSVMHEALHNHYTQKSLSLSP

SEQ ID NO: 88 - protein, 443 aa, synthetic construct
  REGION 1..443: note = an artificially synthesized sequence
QVQLVQSGAEVKKPGASVKVSCKASGYTFTDYEMHWIRQPPGQGLEWIGAIDPKTGDTAYSQKFKGRVTLTADKSTSTAYMELSSLTSEDTAVYYCTRFYSYTYWGQGTLVTVSSASTKGPSVFPLAPSSKSTSGGTAALGCLVEDYFPEPVTVSWNSGALTSGVHTFPAVLESSGLYSLSSVVTVPSSSLGTQTYICNVNHKPSNTKVDEKVEPKSCDKTHTCPPCPAPEAAGGPSVFLFPPKPKDTLMISRTPEVTCVVVDVSHEDPEVKFNWYVDGVEVHNAKTKPREEQYASTYRVVSVLTVLHQDWLNGKEYKCKVSNKALPAPIEKTISKAKGQPREPQVCTLPPSRDELTKNQVSLWCLVKGFYPSDIAVEWESNGQPENNYKTTPPVLDSDGSFFLYSKLTVDKSRWQQGNVFSCSVMHEALHNHYTQKSLSLSP

SEQ ID NO: 89 - protein, 219 aa, synthetic construct
  REGION 1..219: note = an artificially synthesized sequence
DIVMTQSPLSLPVTPGEPASISCRSSQSLVHSNRNTYLHWYQQKPGQAPRLLIYKVSNRFSGVPDRFSGSGSGTDFTLKISRVEAEDVGVYYCSQNTHVPPTFGQGTKLEIKRTVAAPSVFIFPPSDEQLKSGTAKVVCLLNNFYPREAKVQWKVDNALQSGNSKESVTEQDSKDSTYSLSSTLKLSKADYEKHKVYACEVTHQGLSSPVTKSFNRGEC

SEQ ID NO: 90 - protein, 219 aa, synthetic construct
  REGION 1..219: note = an artificially synthesized sequence
DIVMTQSPLSLPVTPGEPASISCRSSQSLVHSNRNTYLHWYQQKPGQAPRLLIYKVSNRFSGVPDRFSGSGSGTDFTLKISRVEAEDVGVYYCSQNTHVPPTFGQGTKLEIKRTVAAPSVFIFPPSDKQLKSGTAKVVCLLNNFYPREAKVQWKVDNALQSGNSKESVTEQDSKDSTYSLSSTLKLSKADYEKHKVYACEVTHQGLSSPVTKSFNRGEC

SEQ ID NO: 91 - protein, 474 aa, synthetic construct
  REGION 1..474: note = an artificially synthesized sequence
MGWSCIILFLVATATGVHSQVQLKQSGPGLVQPSQSLSITCTVSGFSLTNYGVHWVRQSPGKGLEWLGVIWSGGNTDYNTPFTSRLSINKDNSKSQVFFKMNSLQSNDTAIYYCARALTYYDYEFAYWGQGTLVTVSAASTKGPSVFPLAPSSKSTSGGTAALGCLVKDYFPEPVTVSWNSGALTSGVHTFPAVLQSSGLYSLSSVVTVPSSSLGTQTYICNVNHKPSNTKVDKKVEPKSCDKTHTCPPCPAPEAAGGPSVFLFPPKPKDTLMISRTPEVTCVVVDVSHEDPEVKFNWYVDGVEVHNAKTKPREEQYASTYRVVSVLTVLHQDWLNGKEYKCKVSNKALPAPIEKTISKAKGQPREPQVCTLPPSRDELTKNQVSLWCLVKGFYPSDIAVEWESNGQPENNYKTTPPVLDSDGSFFLYSKLTVDKSRWQQGNVFSCSVMHEALHNHYTQKSLSLSPHHHHHHHH

SEQ ID NO: 92 - protein, 233 aa, synthetic construct
  REGION 1..233: note = an artificially synthesized sequence
MGWSCIILFLVATATGVHSDILLTQSPVILSVSPGERVSFSCRASQSIGTNIHWYQQRTNGSPRLLIKYASESISGIPSRFSGSGSGTDFTLSINSVESEDIADYYCQQNNNWPTTFGAGTKLELKRTVAAPSVFIFPPSDEQLKSGTASVVCLLNNFYPREAKVQWKVDNALQSGNSQESVTEQDSKDSTYSLSSTLTLSKADYEKHKVYACEVTHQGLSSPVTKSFNRGEC